European Patent Application EP 4 257 602 A2, published October 11, 2023. Title: Single domain antibodies for complement regulation. Applicant: Aarhus Universitet. The sequence listing filed with the application follows.

SEQUENCE LISTING (85 sequences)

SEQ ID NO: 1 - protein, 1641 aa, Homo sapiens
SPMYSIITPNILRLESEETMVLEAHDAQGDVPVTVTVHDFPGKKLVLSSEKTVLTPATNHMGNVTFTIPANREFKSEKGRNKFVTVQATFGTQVVEKVVLVSLQSGYLFIQTDKTIYTPGSTVLYRIFTVNHKLLPVGRTVMVNIENPEGIPVKQDSLSSQNQLGVLPLSWDIPELVNMGQWKIRAYYENSPQQVFSTEFEVKEYVLPSFEVIVEPTEKFYYIYNEKGLEVTITARFLYGKKVEGTAFVIFGIQDGEQRISLPESLKRIPIEDGSGEVVLSRKVLLDGVQNPRAEDLVGKSLYVSATVILHSGSDMVQAERSGIPIVTSPYQIHFTKTPKYFKPGMPFDLMVFVTNPDGSPAYRVPVAVQGEDTVQSLTQGDGVAKLSINTHPSQKPLSITVRTKKQELSEAEQATRTMQALPYSTVGNSNNYLHLSVLRTELRPGETLNVNFLLRMDRAHEAKIRYYTYLIMNKGRLLKAGRQVREPGQDLVVLPLSITTDFIPSFRLVAYYTLIGASGQREVVADSVWVDVKDSCVGSLVVKSGQSEDRQPVPGQQMTLKIEGDHGARVVLVAVDKGVFVLNKKNKLTQSKIWDVVEKADIGCTPGSGKDYAGVFSDAGLTFTSSSGQQTAQRAELQCPQPAARRRRSVQLTEKRMDKVGKYPKELRKCCEDGMRENPMRFSCQRRTRFISLGEACKKVFLDCCNYITELRRQHARASHLGLARSNLDEDIIAEENIVSRSEFPESWLWNVEDLKEPPKNGISTKLMNIFLKDSITTWEILAVSMSDKKGICVADPFEVTVMQDFFIDLRLPYSVVRNEQVEIRAVLYNYRQNQELKVRVELLHNPAFCSLATTKRRHQQTVTIPPKSSLSVPYVIVPLKTGLQEVEVKAAVYHHFISDGVRKSLKVVPEGIRMNKTVAVRTLDPERLGREGVQKEDIPPADLSDQVPDTESETRILLQGTPVAQMTEDAVDAERLKHLIVTPSGCGEQNMIGMTPTVIAVHYLDETEQWEKFGLEKRQGALELIKKGYTQQLAFRQPSSAFAAFVKRAPSTWLTAYVVKVFSLAVNLIAIDSQVLCGAVKWLILEKQKPDGVFQEDAPVIHQEMIGGLRNNNEKDMALTAFVLISLQEAKDICEEQVNSLPGSITKAGDFLEANYMNLQRSYTVAIAGYALAQMGRLKGPLLNKFLTTAKDKNRWEDPGKQLYNVEATSYALLALLQLKDFDFVPPVVRWLNEQRYYGGGYGSTQATFMVFQALAQYQKDAPDHQELNLDVSLQLPSRSSKITHRIHWESASLLRSEETKENEGFTVTAEGKGQGTLSVVTMYHAKAKDQLTCNKFDLKVTIKPAPETEKRPQDAKNTMILEICTRYRGDQDATMSILDISMMTGFAPDTDDLKQLANGVDRYISKYELDKAFSDRNTLIIYLDKVSHSEDDCLAFKVHQYFNVELIQPGAVKVYAYYNLEESCTRFYHPEKEDGKLNKLCRDELCRCAEENCFIQKSDDKVTLEERLDKACEPGVDYVYKTRLVKVQLSNDFDEYIMAIEQTIKSGSDEVQVGQQRTFISPIKCREALKLEEKKHYLMWGLSSDFWGEKPNLSYIIGKDTWVEHWPEEDECQDEENQKQCQDLGAFTESMVVFGCPN

SEQ ID NO: 2 - protein, 1635 aa, Mus musculus
IPMYSIITPNVLRLESEETIVLEAHDAQGDIPVTVTVQDFLKRQVLTSEKTVLTGASGHLRSVSIKIPASKEFNSDKEGHKYVTVVANFGETVVEKAVMVSFQSGYLFIQTDKTIYTPGSTVLYRIFTVDNNLLPVGKTVVILIETPDGIPVKRDILSSNNQHGILPLSWNIPELVNMGQWKIRAFYEHAPKQIFSAEFEVKEYVLPSFEVRVEPTETFYYIDDPNGLEVSIIAKFLYGKNVDGTAFVIFGVQDGDKKISLAHSLTRVVIEDGVGDAVLTRKVLMEGVRPSNADALVGKSLYVSVTVILHSGSDMVEAERSGIPIVTSPYQIHFTKTPKFFKPAMPFDLMVFVTNPDGSPASKVLVVTQGSNAKALTQDDGVAKLSINTPNSRQPLTITVRTKKDTLPESRQATKTMEAHPYSTMHNSNNYLHLSVSRMELKPGDNLNVNFHLRTDPGHEAKIRYYTYLVMNKGKLLKAGRQVREPGQDLVVLSLPITPEFIPSFRLVAYYTLIGASGQREVVADSVWVDVKDSCIGTLVVKGDPRDNHLAPGQQTTLRIEGNQGARVGLVAVDKGVFVLNKKNKLTQSKIWDVVEKADIGCTPGSGKNYAGVFMDAGLAFKTSQGLQTEQRADLECTKPAASVQLMERRMDKAGQYTDKGLRKCCEDGMRDIPMRYSCQRRARLITQGENCIKAFIDCCNHITKLREQHRRDHVLGLARSELEEDIIPEEDIISRSHFPQSWLWTIEELKEPEKNGISTKVMNIFLKDSITTWEILAVSLSDKKGICVADPYEIRVMQDFFIDLRLPYSVVRNEQVEIRAVLFNYREQEELKVRVELLHNPAFCSMATAKNRYFQTIKIPPKSSVAVPYVIVPLKIGQQEVEVKAAVFNHFISDGVKKTLKVVPEGMRINKTVAIHTLDPEKLGQGGVQKVDVPAADLSDQVPDTDSETRIILQGSPVVQMAEDAVDGERLKHLIVTPAGCGEQNMIGMTPTVIAVHYLDQTEQWEKFGIEKRQEALELIKKGYTQQLAFKQPSSAYAAFNNRPPSTWLTAYVVKVFSLAANLIAIDSHVLCGAVKWLILEKQKPDGVFQEDGPVIHQEMIGGFRNAKEADVSLTAFVLIALQEARDICEGQVNSLPGSINKAGEYIEASYMNLQRPYTVAIAGYALALMNKLEEPYLGKFLNTAKDRNRWEEPDQQLYNVEATSYALLALLLLKDFDSVPPVVRWLNEQRYYGGGYGSTQATFMVFQALAQYQTDVPDHKDLNMDVSFHLPSRSSATTFRLLWENGNLLRSEETKQNEAFSLTAKGKGRGTLSVVAVYHAKLKSKVTCKKFDLRVSIRPAPETAKKPEEAKNTMFLEICTKYLGDVDATMSILDISMMTGFAPDTKDLELLASGVDRYISKYEMNKAFSNKNTLIIYLEKISHTEEDCLTFKVHQYFNVGLIQPGSVKVYSYYNLEESCTRFYHPEKDDGMLSKLCHSEMCRCAEENCFMQQSQEKINLNVRLDKACEPGVDYVYKTELTNIELLDDFDEYTMTIQQVIKSGSDEVQAGQQRKFISHIKCRNALKLQKGKKYLMWGLSSDLWGEKPNTSYIIGKDTWVEHWPEAEECQDQKYQKQCEELGAFTESMVVYGCPN

SEQ ID NO: 3 - protein, 223 aa, Homo sapiens
EDLCRAPDGKKGEAGRPGRRGRPGLKGEQGEPGAPGIRTGIQGLKGDQGEPGPSGNPGKVGYPGPSGPLGARGIPGIKGTKGSPGNIKDQPRPAFSAIRRNPPMGGNVVIFDTVITNQEEPYQNHSGRFVCTVPGYYYFTFQVLSQWEICLSIVSSSRGQVRRSLGFCDTTNKGLFQVVSGGMVLQLQQGDQVWVEKDPKKGHIYQGSEADSVFSGFLIFPSA

SEQ ID NO: 4 - protein, 226 aa, Homo sapiens
QLSCTGPPAIPGIPGIPGTPGPDGQPGTPGIKGEKGLPGLAGDHGEFGEKGDPGIPGNPGKVGPKGPMGPKGGPGAPGAPGPKGESGDYKATQKIAFSATRTINVPLRRDQTIRFDHVITNMNNNYEPRSGKFTCKVPGLYYFTYHASSRGNLCVNLMRGRERAQKVVTFCDYAYNTFQVTTGGMVLKLEQGENVFLQATDKNSLLGMEGANSIFSGFLLFPDMEA

SEQ ID NO: 5 - protein, 217 aa, Homo sapiens
NTGCYGIPGMPGLPGAPGKDGYDGLPGPKGEPGIPAIPGIRGPKGQKGEPGLPGHPGKNGPMGPPGMPGVPGPMGIPGEPGEEGRYKQKFQSVFTVTRQTHQPPAPNSLIRFNAVLTNPQGDYDTSTGKFTCKVPGLYYFVYHASHTANLCVLLYRSGVKVVTFCGHTSKTNQVNSGGVLLRLQVGEEVWLAVNDYYDMVGIQGSDSVFSGFLLFPD

SEQ ID NO: 6 - protein, 767 aa, Homo sapiens
NVNFQKAINEKLGQYASPTAKRCCQDGVTRLPMMRSCEQRAARVQQPDCREPFLSCCQFAESLRKKSRDKGQAGLQRALEILQEEDLIDEDDIPVRSFFPENWLWRVETVDRFQILTLWLPDSLTTWEIHGLSLSKTKGLCVATPVQLRVFREFHLHLRLPMSVRRFEQLELRPVLYNYLDKNLTVSVHVSPVEGLCLAGGGGLAQQVLVPAGSARPVAFSVVPTAAAAVSLKVVARGSFEFPVGDAVSKVLQIEKEGAIHREELVYELNPLDHRGRTLEIPGNSDPNMIPDGDFNSYVRVTASDPLDTLGSEGALSPGGVASLLRLPRGCGEQTMIYLAPTLAASRYLDKTEQWSTLPPETKDHAVDLIQKGYMRIQQFRKADGSYAAWLSRDSSTWLTAFVLKVLSLAQEQVGGSPEKLQETSNWLLSQQQADGSFQDPCPVLDRSMQGGLVGNDETVALTAFVTIALHHGLAVFQDEGAEPLKQRVEASISKANSFLGEKASAGLLGAHAAAITAYALTLTKAPVDLLGVAHNNLMAMAQETGDNLYWGSVTGSQSNAVSPTPAPRNPSDPMPQAPALWIETTAYALLHLLLHEGKAEMADQASAWLTRQGSFQGGFRSTQDTVIALDALSAYWIASHTTEERGLNVTLSSTGRNGFKSHALQLNNRQIRGLEEELQFSLGSKINVKVGGNSKGTLKVLRTYNVLDMKNTTCQDLQIEVTVKGHVEYTMEANEDYEDYEYDELPAKDDPDAPLQPVTPLQLFEG

SEQ ID NO: 7 - protein, 656 aa, Homo sapiens
KPRLLLFSPSVVHLGVPLSVGVQLQDVPRGQVVKGSVFLRNPSRNNVPCSPKVDFTLSSERDFALLSLQVPLKDAKSCGLHQLLRGPEVQLVAHSPWLKDSLSRTTNIQGINLLFSSRRGHLFLQTDQPIYNPGQRVRYRVFALDQKMRPSTDTITVMVENSHGLRVRKKEVYMPSSIFQDDFVIPDISEPGTWKISARFSDGLESNSSTQFEVKKYVLPNFEVKITPGKPYILTVPGHLDEMQLDIQARYIYGKPVQGVAYVRFGLLDEDGKKTFFRGLESQTKLVNGQSHISLSKAEFQDALEKLNMGITDLQGLRLYVAAAIIESPGGEMEEAELTSWYFVSSPFSLDLSKTKRHLVPGAPFLLQALVREMSGSPASGIPVKVSATVSSPGSVPEVQDIQQNTDGSGQVSIPIIIPQTISELQLSVSAGSPHPAIARLTVAAPPSGGPGFLSIERPDSRPPRVGDTLNLNLRAVGSGATFSHYYYMILSRGQIVFMNREPKRTLTSVSVFVDHHLAPSFYFVAFYYHGDHPVANSLRVDVQAGACEGKLELSVDGAKQYRNGESVKLHLETDSLALVALGALDTALYAAGSKSHKPLNMGKVFEAMNSYDLGCGPGGGDSALQVFQAAGLAFSDGDQWTLSRKRLSCPKEKTT

SEQ ID NO: 8 - protein, 291 aa, Homo sapiens
EAPKVVEEQESRVHYTVCIWRNGKVGLSGMAIADVTLLSGFHALRADLEKLTSLSDRYVSHFETEGPHVLLYFDSVPTSRECVGFEAVQEVPVGLVQPASATLYDYYNPERRCSVFYGAPSKSRLLATLCSAEVCQCAEGKCPRQRRALERGLQDEDGYRMKFACYYPRVEYGFQVKVLREDSRAAFRLFETKITQVLHFTKDVKAAANQMRNFLVRASCRLRLEPGKEYLIMGLDGATYDLEGHPQYLLDSNSWIEEMPSERLCRSTRQRAACAQLNDFLQEYGTQGCQV

SEQ ID NO: 9 - protein, 129 aa, Homo sapiens
QVQLVESGGGLVQPGGSLRLSCAASGFTLNQYAIGWFRQAPGKEREGVSCISNSDGGLYYADSVKGRFTISRDNAKNTVYLQMNSLKPEDTAVYYCATDPGGPTMYGSRWCDSRLFYSWGQGTQVTVSS

SEQ ID NO: 10 - protein, 10 aa, unidentified
  REGION 1..10: note = Artificial sequence/unknown
  REGION 1..10: note = MISC_FEATURE - CDR1
GFTLNQYAIG

SEQ ID NO: 11 - protein, 10 aa, unidentified
  REGION 1..10: note = Artificial sequence/unknown
  REGION 1..10: note = MISC_FEATURE - CDR2
CISNSDGGLY

SEQ ID NO: 12 - protein, 20 aa, unidentified
  REGION 1..20: note = Artificial sequence/unknown
  REGION 1..20: note = MISC_FEATURE - CDR3
DPGGPTMYGSRWCDSRLFYS

SEQ ID NO: 13 - protein, 125 aa, unidentified
  REGION 1..125: note = Artificial sequence/unknown
  REGION 1..125: note = MISC_FEATURE - IF75
QVQLVETGGGLVQAGGSLRLSCAASGRTFNNDVMAWFRQAPGTEREFVALITAGGGTHYADSVKGRFVISRDNDKNMAYLQMNSLKSEDTAIYYCGADENPPGWPSRWSSAYDYWGQGTQVTVSS

SEQ ID NO: 14 - protein, 10 aa, unidentified
  REGION 1..10: note = Artificial sequence/unknown
  REGION 1..10: note = MISC_FEATURE - CDR1
GRTFNNDVMA

SEQ ID NO: 15 - protein, 9 aa, unidentified
  REGION 1..9: note = Artificial sequence/unknown
  REGION 1..9: note = MISC_FEATURE - CDR2
LITAGGGTH

SEQ ID NO: 16 - protein, 17 aa, unidentified
  REGION 1..17: note = Artificial sequence/unknown
  REGION 1..17: note = MISC_FEATURE - CDR3
DENPPGWPSRWSSAYDY

SEQ ID NO: 17 - protein, 128 aa, unidentified
  REGION 1..128: note = Artificial sequence/unknown
  REGION 1..128: note = MISC_FEATURE - IF78
QVQLVESGGGLVQDGDSLRLSCAGSGWTFRDSMYNMGWFRQAPGKEREFVAAISWRGGSTLYADSVKGRFTISRDNAKNTVYLQMNSLKPEDTAVYQCAADTSARAALYSTGYEYDHWGQGTQVTVSS

SEQ ID NO: 18 - protein, 12 aa, unidentified
  REGION 1..12: note = Artificial sequence/unknown
  REGION 1..12: note = MISC_FEATURE - CDR1
GWTFRDSMYNMG

SEQ ID NO: 19 - protein, 11 aa, unidentified
  REGION 1..11: note = Artificial sequence/unknown
  REGION 1..11: note = MISC_FEATURE - CDR2
AISWRGGSTLY

SEQ ID NO: 20 - protein, 17 aa, unidentified
  REGION 1..17: note = Artificial sequence/unknown
  REGION 1..17: note = MISC_FEATURE - CDR3
DTSARAALYSTGYEYDH

SEQ ID NO: 21 - protein, 127 aa, unidentified
  REGION 1..127: note = Artificial sequence/unknown
  REGION 1..127: note = MISC_FEATURE - IH31
QVQLVESGGGLVQAGGSLRLSCAASGRTSSDHITAWFRQAPGKEREFVASINWSGSRAYYADSDKRRFTISRDNAKNTVSLQTNSLKPEDTAVYYCAVKFADISDAYYHHQTDYDYWGQGTQVTVSS

SEQ ID NO: 22 - protein, 10 aa, unidentified
  REGION 1..10: note = Artificial sequence/unknown
  REGION 1..10: note = MISC_FEATURE - CDR1
GRTSSDHITA

SEQ ID NO: 23 - protein, 10 aa, unidentified
  REGION 1..10: note = Artificial sequence/unknown
  REGION 1..10: note = MISC_FEATURE - CDR2
SINWSGSRAY

SEQ ID NO: 24 - protein, 18 aa, unidentified
  REGION 1..18: note = Artificial sequence/unknown
  REGION 1..18: note = MISC_FEATURE - CDR3
KFADISDAYYHHQTDYDY

SEQ ID NO: 25 - protein, 119 aa, unidentified
  REGION 1..119: note = Artificial sequence/unknown
  REGION 1..119: note = MISC_FEATURE - IH33
QVQLVETGGGLVQTGGSLRLSCAASGSTDSIAAIIWYRQTPENEREFVAGITSGVNTNYAAPVKGRFTISRDNAKNTVYLQMNSLKPEDTGVYYCKAAVVMGPSTTDYWGQGTQVTVSS

SEQ ID NO: 26 - protein, 10 aa, unidentified
  REGION 1..10: note = Artificial sequence/unknown
  REGION 1..10: note = MISC_FEATURE - CDR1
GSTDSIAAII

SEQ ID NO: 27 - protein, 7 aa, unidentified
  REGION 1..7: note = Artificial sequence/unknown
  REGION 1..7: note = MISC_FEATURE - CDR2
GITSGVN

SEQ ID NO: 28 - protein, 11 aa, unidentified
  REGION 1..11: note = Artificial sequence/unknown
  REGION 1..11: note = MISC_FEATURE - CDR3
AVVMGPSTTDY

SEQ ID NO: 29 - protein, 124 aa, unidentified
  REGION 1..124: note = Artificial sequence/unknown
  REGION 1..124: note = MISC_FEATURE - IH35
QVQLVETGGGVAQAGGSLRLSCAASGFSFDDYAIGWLRQAPGKEREGVSCISAGDGSPQYADSVKGRFTISSDNAKNTVYLQMNSLKPEDTAVYYCAVSRWSNCAWDYYGMDPWGKGTLVTVSS

SEQ ID NO: 30 - protein, 10 aa, unidentified
  REGION 1..10: note = Artificial sequence/unknown
  REGION 1..10: note = MISC_FEATURE - CDR1
GFSFDDYAIG

SEQ ID NO: 31 - protein, 10 aa, unidentified
  REGION 1..10: note = Artificial sequence/unknown
  REGION 1..10: note = MISC_FEATURE - CDR2
CISAGDGSPQ

SEQ ID NO: 32 - protein, 15 aa, unidentified
  REGION 1..15: note = Artificial sequence/unknown
  REGION 1..15: note = MISC_FEATURE - CDR3
SRWSNCAWDYYGMDP

SEQ ID NO: 33 - protein, 125 aa, unidentified
  REGION 1..125: note = Artificial sequence/unknown
  REGION 1..125: note = MISC_FEATURE - IH37
QVQLVESGGGLAQAGGSLRLSCQGSGRTFNNDVLAWFRQAPGKEREYVAMITSGGNPFYADSVKGRFVISRDNDKNTVYLQMNSLKSEDTAIYYCAADENPPGWPSRWSSAYDYWGQGTQVTVSS

SEQ ID NO: 34 - protein, 10 aa, unidentified
  REGION 1..10: note = Artificial sequence/unknown
  REGION 1..10: note = MISC_FEATURE - CDR1
GRTFNNDVLA

SEQ ID NO: 35 - protein, 9 aa, unidentified
  REGION 1..9: note = Artificial sequence/unknown
  REGION 1..9: note = MISC_FEATURE - CDR2
MITSGGNPF

SEQ ID NO: 36 - protein, 17 aa, unidentified
  REGION 1..17: note = Artificial sequence/unknown
  REGION 1..17: note = MISC_FEATURE - CDR3
DENPPGWPSRWSSAYDY

SEQ ID NO: 37 - protein, 124 aa, unidentified
  REGION 1..124: note = Artificial sequence/unknown
  REGION 1..124: note = MISC_FEATURE - IH39
QVQLVESGGGLVQAGGSLRLSCVAYGVASVTTVMGWFRQSPGKEREFVAAIGPSGGTHYGDSAKGRFTISRDNAKNTVYLQMNSLKPEDTAVYDCAADLRGGGMWASSGRYEYWGQGTQVTVSS

SEQ ID NO: 38 - protein, 10 aa, unidentified
  REGION 1..10: note = Artificial sequence/unknown
  REGION 1..10: note = MISC_FEATURE - CDR1
GVASVTTVMG

SEQ ID NO: 39 - protein, 9 aa, unidentified
  REGION 1..9: note = Artificial sequence/unknown
  REGION 1..9: note = MISC_FEATURE - CDR2
AIGPSGGTH

SEQ ID NO: 40 - protein, 16 aa, unidentified
  REGION 1..16: note = Artificial sequence/unknown
  REGION 1..16: note = MISC_FEATURE - CDR3
DLRGGGMWASSGRYEY

SEQ ID NO: 41 - protein, 124 aa, unidentified
  REGION 1..124: note = Artificial sequence/unknown
  REGION 1..124: note = MISC_FEATURE - hC4bNb6
QVQLVETGGGVVRAGGSLRLSCAASGRTLGRYSMAWFRQAPGKERQFVAAINWSGGSTYYPDFAKDRFTISRDSAKNMVYLQMNSLKPEDTAVYYCAAGGMDIEITRANEYDYWGQGTQVTVSS

SEQ ID NO: 42 - protein, 10 aa, unidentified
  REGION 1..10: note = Artificial sequence/unknown
  REGION 1..10: note = MISC_FEATURE - CDR1
GRTLGRYSMA

SEQ ID NO: 43 - protein, 10 aa, unidentified
  REGION 1..10: note = Artificial sequence/unknown
  REGION 1..10: note = MISC_FEATURE - CDR2
AINWSGGSTY

SEQ ID NO: 44 - protein, 15 aa, unidentified
  REGION 1..15: note = Artificial sequence/unknown
  REGION 1..15: note = MISC_FEATURE - CDR3
GGMDIEITRANEYDY

SEQ ID NO: 45 - protein, 124 aa, unidentified
  REGION 1..124: note = Artificial sequence/unknown
  REGION 1..124: note = MISC_FEATURE - hC4Nb8
QVQLVESGGGLVQTGDSLRLSCAASGRTFSRYAMGWFRQAPGKERELVAAINWSGGSTYYADFAKGRFTISRDNAKNMLYLRMSSLKPEDTAVYYCAAGGPEVEITRANEYDYWGQGTQVTVSS

SEQ ID NO: 46 - protein, 10 aa, unidentified
  REGION 1..10: note = Artificial sequence/unknown
  REGION 1..10: note = MISC_FEATURE - CDR1
GRTFSRYAMG

SEQ ID NO: 47 - protein, 10 aa, unidentified
  REGION 1..10: note = Artificial sequence/unknown
  REGION 1..10: note = MISC_FEATURE - CDR2
AINWSGGSTY

SEQ ID NO: 48 - protein, 15 aa, unidentified
  REGION 1..15: note = Artificial sequence/unknown
  REGION 1..15: note = MISC_FEATURE - CDR3
GGPEVEITRANEYDY

SEQ ID NO: 49 - protein, 118 aa, unidentified [sequence omitted]

SEQ ID NO: 50 - protein, 11 aa, unidentified
  REGION 1..11: note = Artificial sequence/unknown
  REGION 1..11: note = MISC_FEATURE - CDR1
SGSTFSDYAMG

SEQ ID NO: 51 - protein, 9 aa, unidentified
  REGION 1..9: note = Artificial sequence/unknown
  REGION 1..9: note = MISC_FEATURE - CDR2
AIYSTGRTN

SEQ ID NO: 52 - protein, 10 aa, unidentified
  REGION 1..10: note = Artificial sequence/unknown
  REGION 1..10: note = MISC_FEATURE - CDR3
LGATTMINTK

SEQ ID NO: 53 - protein, 128 aa, unidentified
  REGION 1..128: note = Artificial sequence/unknown
  REGION 1..128: note = MISC_FEATURE - DI62
QVQLVESGGGLVQAGGSLRLSCAASGRTFSDYTMGWFRQAPGKEREFVAGLSTGGSFTRYAASVEGRFTISRDNAKTTVYLQMNNLQPEDTAVYYCAADFTPYGTNWSRFREARDHYWGQGTQVTVSS

SEQ ID NO: 54 - protein, 11 aa, unidentified
  REGION 1..11: note = Artificial sequence/unknown
  REGION 1..11: note = MISC_FEATURE - CDR1
SGRTFSDYTMG

SEQ ID NO: 55 - protein, 10 aa, unidentified
  REGION 1..10: note = Artificial sequence/unknown
  REGION 1..10: note = MISC_FEATURE - CDR2
GLSTGGSFTR

SEQ ID NO: 56 - protein, 19 aa, unidentified
  REGION 1..19: note = Artificial sequence/unknown
  REGION 1..19: note = MISC_FEATURE - CDR3
DFTPYGTNWSRFREARDHY

SEQ ID NO: 57 - protein, 127 aa, unidentified
  REGION 1..127: note = Artificial sequence/unknown
  REGION 1..127: note = MISC_FEATURE - EWE-hC3Nb1
MEWEQVQLVETGGGLVQAGGSLRLSCAASGSIFSINAMGWFRQAPGKEREFVATINRSGGRTYYADSVKGRFTISRDNGKNMVYLQMHSLKPEDTAIYYCAAGTGWSPQTDNEYNYWGQGTQVTVSS

SEQ ID NO: 58 - protein, 11 aa, unidentified
  REGION 1..11: note = Artificial sequence/unknown
  REGION 1..11: note = MISC_FEATURE - CDR1
SGSIFSINAMG

SEQ ID NO: 59 - protein, 10 aa, unidentified
  REGION 1..10: note = Artificial sequence/unknown
  REGION 1..10: note = MISC_FEATURE - CDR2
TINRSGGRTY

SEQ ID NO: 60 - protein, 14 aa, unidentified
  REGION 1..14: note = Artificial sequence/unknown
  REGION 1..14: note = MISC_FEATURE - CDR3
GTGWSPQTDNEYNY

SEQ ID NO: 61 - protein, 358 aa, unidentified
  REGION 1..358: note = Artificial sequence/unknown
  REGION 1..358: note = MISC_FEATURE - IgG-Fc-hC3Nb1
APLEPKSSDKTHTCPPCPAPELLGGPSVFLFPPKPKDTLMISRTPEVTCVVVDVSHEDPEVKFNWYVDGVEVHNAKTKPREEQYNSTYRVVSVLTVLHQDWLNGKEYKCKVSNKALPAPIEKTISKAKGQPREPQVYTLPPSREEMTKNQVSLTCLVKGFYPSDIAVEWESNGQPENNYKTTPPVLDSDGSFFLYSKLTVDKSRWQQGNVFSCSVMHEALHNHYTQKSLSLSPGAQVQLVETGGGLVQAGGSLRLSCAASGSIFSINAMGWFRQAPGKEREFVATINRSGGRTYYADSVKGRFTISRDNGKNMVYLQMHSLKPEDTAIYYCAAGTGWSPQTDNEYNYWGQGTQVTVSS

SEQ ID NO: 62 - protein, 11 aa, unidentified
  REGION 1..11: note = Artificial sequence/unknown
  REGION 1..11: note = MISC_FEATURE - CDR1
SGSIFSINAMG

SEQ ID NO: 63 - protein, 10 aa, unidentified
  REGION 1..10: note = Artificial sequence/unknown
  REGION 1..10: note = MISC_FEATURE - CDR2
TINRSGGRTY

SEQ ID NO: 64 - protein, 14 aa, unidentified
  REGION 1..14: note = Artificial sequence/unknown
  REGION 1..14: note = MISC_FEATURE - CDR3
GTGWSPQTDNEYNY

SEQ ID NO: 65 - protein, 10 aa, synthetic construct
  REGION 1..10: note = Artificial sequence/unknown
  REGION 1..10: note = MISC_FEATURE - polypeptide linker
GGGGSGGGGS

SEQ ID NO: 66 - protein, 129 aa, unidentified
  REGION 1..129: note = Artificial sequence/unknown
  REGION 1..129: note = MISC_FEATURE - hC4Nb5
QVQLVETGGGLVQPGGSLRLSCAASGRTFNKNPMAWFRQPPGQERDLVAAISWSGDSTNYANSVQGRFTISRNNAQRTVSLSMNNLKPEDTAVYYCAAVGRTDYSPNSLALTAQNYDYWGQGTQVTVSS

SEQ ID NO: 67 - protein, 10 aa, unidentified
  REGION 1..10: note = Artificial sequence/unknown
  REGION 1..10: note = MISC_FEATURE - CDR1
GRTFNKNPMA

SEQ ID NO: 68 - protein, 10 aa, unidentified
  REGION 1..10: note = Artificial sequence/unknown
  REGION 1..10: note = MISC_FEATURE - CDR2
AISWSGDSTN

SEQ ID NO: 69 - protein, 19 aa, unidentified
  REGION 1..19: note = Artificial sequence/unknown
  REGION 1..19: note = MISC_FEATURE - CDR3
VGRTDYSPNSLALTAQNYD

SEQ ID NO: 70 - protein, 124 aa, unidentified
  REGION 1..124: note = Artificial sequence/unknown
  REGION 1..124: note = MISC_FEATURE - hC4Nb4
QVQLVETGGGLVEAGGSLRISCAASGRYAMGWFRQAPGNERDFVAAISRSGDSANYADTAWGRFTISRDNAQNTMTLQMNSLKPEDTAVYYCAAKAGLYSLNSLFLRSQEYTYWGQGTQVTVSS

SEQ ID NO: 71 - protein, 6 aa, unidentified
  REGION 1..6: note = Artificial sequence/unknown
  REGION 1..6: note = MISC_FEATURE - CDR1
GRYAMG

SEQ ID NO: 72 - protein, 10 aa, unidentified
  REGION 1..10: note = Artificial sequence/unknown
  REGION 1..10: note = MISC_FEATURE - CDR2
AISRSGDSAN

SEQ ID NO: 73 - protein, 19 aa, unidentified
  REGION 1..19: note = Artificial sequence/unknown
  REGION 1..19: note = MISC_FEATURE - CDR3
KAGLYSLNSLFLRSQEYTY

SEQ ID NO: 74 - protein, 148 aa, Mus musculus [sequence omitted]

SEQ ID NO: 75 - protein, 45 aa, Mus musculus
EKINLNVRLDKACPEAEECQDQKYQKQCEELGAFTESMVVYGCPN

SEQ ID NO: 76 - protein, 126 aa, unidentified
  REGION 1..126: note = Artificial sequence/unknown
  REGION 1..126: note = MISC_FEATURE - pNSL270
QVQLVESGGGLVQAGGSLRLSCVASASTLDIYTYAMAWFRQAPGKRREFVAAISRNGYSTYYADSVKGRFTISKLNAKNTLYLQMNSLEPEDTAAYYCAADRTTEVVDREDDYGYWGQGTQVTVSS

SEQ ID NO: 77 - protein, 12 aa, unidentified
  REGION 1..12: note = Artificial sequence/unknown
  REGION 1..12: note = MISC_FEATURE - CDR1
ASTLDIYTYAMA

SEQ ID NO: 78 - protein, 10 aa, unidentified
  REGION 1..10: note = Artificial sequence/unknown
  REGION 1..10: note = MISC_FEATURE - CDR2
AISRNGYSTY

SEQ ID NO: 79 - protein, 15 aa, unidentified
  REGION 1..15: note = Artificial sequence/unknown
  REGION 1..15: note = MISC_FEATURE - CDR3
DRTTEVVDREDDYGY

SEQ ID NO: 80 - protein, 767 aa, Homo sapiens
NVNFQKAINEKLGQYASPTAKRCCQDGVTRLPMMRSCEQRAARVQQPDCREPFLSCCQFAESLRKKSRDKGQAGLQRALEILQEEDLIDEDDIPVRSFFPENWLWRVETVDRFQILTLWLPDSLTTWEIHGLSLSKTKGLCVATPVQLRVFREFHLHLRLPMSVRRFEQLELRPVLYNYLDKNLTVSVHVSPVEGLCLAGGGGLAQQVLVPAGSARPVAFSVVPTAATAVSLKVVARGSFEFPVGDAVSKVLQIEKEGAIHREELVYELNPLDHRGRTLEIPGNSDPNMIPDGDFNSYVRVTASDPLDTLGSEGALSPGGVASLLRLPRGCGEQTMIYLAPTLAASRYLDKTEQWSTLPPETKDHAVDLIQKGYMRIQQFRKADGSYAAWLSRGSSTWLTAFVLKVLSLAQEQVGGSPEKLQETSNWLLSQQQADGSFQDLSPVIHRSMQGGLVGNDETVALTAFVTIALHHGLAVFQDEGAEPLKQRVEASISKASSFLGEKASAGLLGAHAAAITAYALTLTKAPADLRGVAHNNLMAMAQETGDNLYWGSVTGSQSNAVSPTPAPRNPSDPMPQAPALWIETTAYALLHLLLHEGKAEMADQAAAWLTRQGSFQGGFRSTQDTVIALDALSAYWIASHTTEERGLNVTLSSTGRNGFKSHALQLNNRQIRGLEEELQFSLGSKINVKVGGNSKGTLKVLRTYNVLDMKNTTCQDLQIEVTVKGHVEYTMEANEDYEDYEYDELPAKDDPDAPLQPVTPLQLFEG

SEQ ID NO: 81 - protein, 690 aa, Homo sapiens
ALEILQEEDLIDEDDIPVRSFFPENWLWRVETVDRFQILTLWLPDSLTTWEIHGLSLSKTKGLCVATPVQLRVFREFHLHLRLPMSVRRFEQLELRPVLYNYLDKNLTVSVHVSPVEGLCLAGGGGLAQQVLVPAGSARPVAFSVVPTAAAAVSLKVVARGSFEFPVGDAVSKVLQIEKEGAIHREELVYELNPLDHRGRTLEIPGNSDPNMIPDGDFNSYVRVTASDPLDTLGSEGALSPGGVASLLRLPRGCGEQTMIYLAPTLAASRYLDKTEQWSTLPPETKDHAVDLIQKGYMRIQQFRKADGSYAAWLSRDSSTWLTAFVLKVLSLAQEQVGGSPEKLQETSNWLLSQQQADGSFQDPCPVLDRSMQGGLVGNDETVALTAFVTIALHHGLAVFQDEGAEPLKQRVEASISKANSFLGEKASAGLLGAHAAAITAYALTLTKAPVDLLGVAHNNLMAMAQETGDNLYWGSVTGSQSNAVSPTPAPRNPSDPMPQAPALWIETTAYALLHLLLHEGKAEMADQASAWLTRQGSFQGGFRSTQDTVIALDALSAYWIASHTTEERGLNVTLSSTGRNGFKSHALQLNNRQIRGLEEELQFSLGSKINVKVGGNSKGTLKVLRTYNVLDMKNTTCQDLQIEVTVKGHVEYTMEANEDYEDYEYDELPAKDDPDAPLQPVTPLQLFEG

SEQ ID NO: 82 - protein, 690 aa, Homo sapiens
ALEILQEEDLIDEDDIPVRSFFPENWLWRVETVDRFQILTLWLPDSLTTWEIHGLSLSKTKGLCVATPVQLRVFREFHLHLRLPMSVRRFEQLELRPVLYNYLDKNLTVSVHVSPVEGLCLAGGGGLAQQVLVPAGSARPVAFSVVPTAATAVSLKVVARGSFEFPVGDAVSKVLQIEKEGAIHREELVYELNPLDHRGRTLEIPGNSDPNMIPDGDFNSYVRVTASDPLDTLGSEGALSPGGVASLLRLPRGCGEQTMIYLAPTLAASRYLDKTEQWSTLPPETKDHAVDLIQKGYMRIQQFRKADGSYAAWLSRGSSTWLTAFVLKVLSLAQEQVGGSPEKLQETSNWLLSQQQADGSFQDLSPVIHRSMQGGLVGNDETVALTAFVTIALHHGLAVFQDEGAEPLKQRVEASISKASSFLGEKASAGLLGAHAAAITAYALTLTKAPADLRGVAHNNLMAMAQETGDNLYWGSVTGSQSNAVSPTPAPRNPSDPMPQAPALWIETTAYALLHLLLHEGKAEMADQAAAWLTRQGSFQGGFRSTQDTVIALDALSAYWIASHTTEERGLNVTLSSTGRNGFKSHALQLNNRQIRGLEEELQFSLGSKINVKVGGNSKGTLKVLRTYNVLDMKNTTCQDLQIEVTVKGHVEYTMEANEDYEDYEYDELPAKDDPDAPLQPVTPLQLFEG

SEQ ID NO: 83 - protein, 654 aa, Mus musculus
KPRLLLFSPSVVNLGTPLSVGVQLLDAPPGQEVKGSVFLRNPKGGSCSPKKDFKLSSGDDFVLLSLEVPLEDVRSCGLFDLRRAPHIQLVAQSPWLRNTAFKATETQGVNLLFSSRRGHIFVQTDQPIYNPGQRVRYRVFALDQKMRPSTDFLTITVENSHGLRVLKKEIFTSTSIFQDAFTIPDISEPGTWKISARFSDGLESNRSTHFEVKKYVLPNFEVKITPWKPYILMVPSNSDEIQLDIQARYIYGKPVQGVAYTRFALMDEQGKRTFLRGLETQAKLVEGRTHISISKDQFQAALDKINIGVRDLEGLRLYAATAVIESPGGEMEEAELTSWRFVSSAFSLDLSRTKRHLVPGAHFLLQALVQEMSGSEASNVPVKVSATLVSGSDSQVLDIQQSTNGIGQVSISFPIPPTVTELRLLVSAGSLYPAIARLTVQAPPSRGTGFLSIEPLDPRSPSVGDTFILNLQPVGIPAPTFSHYYYMIISRGQIMAMGREPRKTVTSVSVLVDHQLAPSFYFVAYFYHQGHPVANSLLINIQSRDCEGKLQLKVDGAKEYRNADMMKLRIQTDSKALVALGAVDMALYAVGGRSHKPLDMSKVFEVINSYNVGCGPGGGDDALQVFQDAGLAFSDGDRLTQTREDLSCPKEKKS

SEQ ID NO: 84 - protein, 766 aa, Mus musculus
NVNFQKAVSEKLGQYSSPDAKRCCQDGMTKLPMKRTCEQRAARVPQQACREPFLSCCKFAEDLRRNQTRSQAHLARNNHNMLQEEDLIDEDDILVRTSFPENWLWRVEPVDSSKLLTVWLPDSMTTWEIHGVSLSKSKGLCVAKPTRVRVFRKFHLHLRLPISIRRFEQFELRPVLYNYLNDDVAVSVHVTPVEGLCLAGGGMMAQQVTVPAGSARPVAFSVVPTAAANVPLKVVARGVFDLGDAVSKILQIEKEGAIHREELVYNLDPLNNLGRTLEIPGSSDPNIVPDGDFSSLVRVTASEPLETMGSEGALSPGGVASLLRLPQGCAEQTMIYLAPTLTASNYLDRTEQWSKLSPETKDHAVDLIQKGYMRIQQFRKNDGSFGAWLHRDSSTWLTAFVLKILSLAQEQVGNSPEKLQETASWLLAQQLGDGSFHDPCPVIHRAMQGGLVGSDETVALTAFVVIALHHGLDVFQDDDAKQLKNRVEASITKANSFLGQKASAGLLGAHAAAITAYALTLTKASEDLRNVAHNSLMAMAEETGEHLYWGLVLGSQDKVVLRPTAPRSPTEPVPQAPALWIETTAYALLHLLLREGKGKMADKAASWLTHQGSFHGAFRSTQDTVVTLDALSAYWIASHTTEEKALNVTLSSMGRNGLKTHGLHLNNHQVKGLEEELKFSLGSTISVKVEGNSKGTLKILRTYNVLDMKNTTCQDLQIEVKVTGAVEYAWDANEDYEDYYDMPAADDPSVPLQPVTPLQLFEGRRS

SEQ ID NO: 85 - protein, 291 aa, Mus musculus
EAPKVVEEQESRVQYTVCIWRNGKLGLSGMAIADITLLSGFHALRADLEKLTSLSDRYVSHFETDGPHVLLYFDSVPTTRECVGFGASQEVVVGLVQPSSAVLYDYYSPDHKCSVFYAAPTKSQLLATLCSGDVCQCAEGKCPRLLRSLERRVEDKDGYRMRFACYYPRVEYGFTVKVLREDGRAAFRLFESKITQVLHFRKDTMASIGQTRNFLSRASCRLRLEPNKEYLIMGMDGETSDNKGDPQYLLDSNTWIEEMPSEQMCKSTRHRAACFQLKDFLMEFSSRGCQV